European Patent Application EP 4 524 265 A2, published March 19, 2025. Title: COMPOSITIONS AND METHODS FOR QUANTIFYING A NUCLEIC ACID SEQUENCE IN A SAMPLE. Applicant: Envirologix, Inc. Application EP. The sequence listing filed with the application follows.

SEQUENCE LISTING (61 sequences)

SEQ ID NO: 1 - DNA, 33 bp, synthetic construct
  misc_feature 1..33: note = Description of Artificial Sequence: Synthetic oligonucleotide
  misc_feature 1..33: note = Description of Combined DNA/RNA Molecule: Synthetic oligonucleotide
  modified_base 22: mod_base = OTHER; note = 2'-O-methyl modified RNA base
  source 1..33: mol_type = other DNA
  misc_difference 1..33: note = DNA or RNA
tgactccatatggagtcacatggttcattcgtg

SEQ ID NO: 2 - DNA, 33 bp, synthetic construct; identical to SEQ ID NO: 1
  misc_feature 1..33: note = Description of Artificial Sequence: Synthetic oligonucleotide
  misc_feature 1..33: note = Description of Combined DNA/RNA Molecule: Synthetic oligonucleotide
  modified_base 23: mod_base = OTHER; note = 2'-O-methyl modified RNA base
  source 1..33: mol_type = other DNA
  misc_difference 1..33: note = DNA or RNA

SEQ ID NO: 3 - DNA, 33 bp, synthetic construct; identical to SEQ ID NO: 1
  misc_feature 1..33: note = Description of Artificial Sequence: Synthetic oligonucleotide
  misc_feature 1..33: note = Description of Combined DNA/RNA Molecule: Synthetic oligonucleotide
  modified_base 24: mod_base = OTHER; note = 2'-O-methyl modified RNA base
  source 1..33: mol_type = other DNA
  misc_difference 1..33: note = DNA or RNA

SEQ ID NO: 4 - DNA, 33 bp, synthetic construct; identical to SEQ ID NO: 1
  misc_feature 1..33: note = Description of Artificial Sequence: Synthetic oligonucleotide
  misc_feature 1..33: note = Description of Combined DNA/RNA Molecule: Synthetic oligonucleotide
  modified_base 25: mod_base = OTHER; note = 2'-O-methyl modified RNA base
  source 1..33: mol_type = other DNA
  misc_difference 1..33: note = DNA or RNA

SEQ ID NO: 5 - DNA, 33 bp, synthetic construct; identical to SEQ ID NO: 1
  misc_feature 1..33: note = Description of Artificial Sequence: Synthetic oligonucleotide
  misc_feature 1..33: note = Description of Combined DNA/RNA Molecule: Synthetic oligonucleotide
  modified_base 26: mod_base = OTHER; note = 2'-O-methyl modified RNA base
  source 1..33: mol_type = other DNA
  misc_difference 1..33: note = DNA or RNA

SEQ ID NO: 6 - DNA, 33 bp, synthetic construct; identical to SEQ ID NO: 1
  misc_feature 1..33: note = Description of Artificial Sequence: Synthetic oligonucleotide
  misc_feature 1..33: note = Description of Combined DNA/RNA Molecule: Synthetic oligonucleotide
  modified_base 27: mod_base = OTHER; note = 2'-O-methyl modified RNA base
  source 1..33: mol_type = other DNA
  misc_difference 1..33: note = DNA or RNA

SEQ ID NO: 7 - DNA, 33 bp, synthetic construct; identical to SEQ ID NO: 1
  misc_feature 1..33: note = Description of Artificial Sequence: Synthetic oligonucleotide
  misc_feature 1..33: note = Description of Combined DNA/RNA Molecule: Synthetic oligonucleotide
  modified_base 28: mod_base = OTHER; note = 2'-O-methyl modified RNA base
  source 1..33: mol_type = other DNA
  misc_difference 1..33: note = DNA or RNA

SEQ ID NO: 8 - DNA, 33 bp, synthetic construct; identical to SEQ ID NO: 1
  misc_feature 1..33: note = Description of Artificial Sequence: Synthetic oligonucleotide
  misc_feature 1..33: note = Description of Combined DNA/RNA Molecule: Synthetic oligonucleotide
  modified_base 29: mod_base = OTHER; note = 2'-O-methyl modified RNA base
  source 1..33: mol_type = other DNA
  misc_difference 1..33: note = DNA or RNA

SEQ ID NO: 9 - DNA, 33 bp, synthetic construct; identical to SEQ ID NO: 1
  misc_feature 1..33: note = Description of Artificial Sequence: Synthetic oligonucleotide
  misc_feature 1..33: note = Description of Combined DNA/RNA Molecule: Synthetic oligonucleotide
  modified_base 30: mod_base = OTHER; note = 2'-O-methyl modified RNA base
  source 1..33: mol_type = other DNA
  misc_difference 1..33: note = DNA or RNA

SEQ ID NO: 10 - DNA, 33 bp, synthetic construct; identical to SEQ ID NO: 1
  misc_feature 1..33: note = Description of Artificial Sequence: Synthetic oligonucleotide
  misc_feature 1..33: note = Description of Combined DNA/RNA Molecule: Synthetic oligonucleotide
  modified_base 31: mod_base = OTHER; note = 2'-O-methyl modified RNA base
  source 1..33: mol_type = other DNA
  misc_difference 1..33: note = DNA or RNA

SEQ ID NO: 11 - DNA, 33 bp, synthetic construct; identical to SEQ ID NO: 1
  misc_feature 1..33: note = Description of Artificial Sequence: Synthetic oligonucleotide
  misc_feature 1..33: note = Description of Combined DNA/RNA Molecule: Synthetic oligonucleotide
  modified_base 32: mod_base = OTHER; note = 2'-O-methyl modified RNA base
  source 1..33: mol_type = other DNA
  misc_difference 1..33: note = DNA or RNA

SEQ ID NO: 12 - DNA, 33 bp, synthetic construct; identical to SEQ ID NO: 1
  misc_feature 1..33: note = Description of Artificial Sequence: Synthetic oligonucleotide
  misc_feature 1..33: note = Description of Combined DNA/RNA Molecule: Synthetic oligonucleotide
  modified_base 33: mod_base = OTHER; note = 2'-O-methyl modified RNA base
  source 1..33: mol_type = other DNA
  misc_difference 1..33: note = DNA or RNA

SEQ ID NO: 13 - DNA, 33 bp, synthetic construct; identical to SEQ ID NO: 1
  misc_feature 1..33: note = Description of Artificial Sequence: Synthetic oligonucleotide
  misc_feature 1..33: note = Description of Combined DNA/RNA Molecule: Synthetic oligonucleotide
  modified_base 22..23: mod_base = OTHER; note = 2'-O-methyl modified RNA base
  source 1..33: mol_type = other DNA
  misc_difference 1..33: note = DNA or RNA

SEQ ID NO: 14 - DNA, 33 bp, synthetic construct; identical to SEQ ID NO: 1
  misc_feature 1..33: note = Description of Artificial Sequence: Synthetic oligonucleotide
  misc_feature 1..33: note = Description of Combined DNA/RNA Molecule: Synthetic oligonucleotide
  modified_base 23..24: mod_base = OTHER; note = 2'-O-methyl modified RNA base
  source 1..33: mol_type = other DNA
  misc_difference 1..33: note = DNA or RNA

SEQ ID NO: 15 - DNA, 33 bp, synthetic construct
  misc_feature 1..33: note = Description of Artificial Sequence: Synthetic oligonucleotide
  misc_feature 1..33: note = Description of Combined DNA/RNA Molecule: Synthetic oligonucleotide
  modified_base 24..25: mod_base = OTHER; note = 2'-O-methyl modified RNA base
  source 1..33: mol_type = other DNA
  misc_difference 1..33: note = DNA or RNA
tgactccatatggagtcacatggtcattcgtgt

SEQ ID NO: 16 - DNA, 33 bp, synthetic construct; identical to SEQ ID NO: 1
  misc_feature 1..33: note = Description of Artificial Sequence: Synthetic oligonucleotide
  misc_feature 1..33: note = Description of Combined DNA/RNA Molecule: Synthetic oligonucleotide
  modified_base 25..26: mod_base = OTHER; note = 2'-O-methyl modified RNA base
  source 1..33: mol_type = other DNA
  misc_difference 1..33: note = DNA or RNA

SEQ ID NO: 17 - DNA, 33 bp, synthetic construct; identical to SEQ ID NO: 1
  misc_feature 1..33: note = Description of Artificial Sequence: Synthetic oligonucleotide
  misc_feature 1..33: note = Description of Combined DNA/RNA Molecule: Synthetic oligonucleotide
  modified_base 26..27: mod_base = OTHER; note = 2'-O-methyl modified RNA base
  source 1..33: mol_type = other DNA
  misc_difference 1..33: note = DNA or RNA

SEQ ID NO: 18 - DNA, 33 bp, synthetic construct; identical to SEQ ID NO: 1
  misc_feature 1..33: note = Description of Artificial Sequence: Synthetic oligonucleotide
  misc_feature 1..33: note = Description of Combined DNA/RNA Molecule: Synthetic oligonucleotide
  modified_base 27..28: mod_base = OTHER; note = 2'-O-methyl modified RNA base
  source 1..33: mol_type = other DNA
  misc_difference 1..33: note = DNA or RNA

SEQ ID NO: 19 - DNA, 33 bp, synthetic construct; identical to SEQ ID NO: 1
  misc_feature 1..33: note = Description of Artificial Sequence: Synthetic oligonucleotide
  misc_feature 1..33: note = Description of Combined DNA/RNA Molecule: Synthetic oligonucleotide
  modified_base 28..29: mod_base = OTHER; note = 2'-O-methyl modified RNA base
  source 1..33: mol_type = other DNA
  misc_difference 1..33: note = DNA or RNA

SEQ ID NO: 20 - DNA, 33 bp, synthetic construct; identical to SEQ ID NO: 1
  misc_feature 1..33: note = Description of Artificial Sequence: Synthetic oligonucleotide
  misc_feature 1..33: note = Description of Combined DNA/RNA Molecule: Synthetic oligonucleotide
  modified_base 29..30: mod_base = OTHER; note = 2'-O-methyl modified RNA base
  source 1..33: mol_type = other DNA
  misc_difference 1..33: note = DNA or RNA

SEQ ID NO: 21 - DNA, 33 bp, synthetic construct; identical to SEQ ID NO: 1
  misc_feature 1..33: note = Description of Artificial Sequence: Synthetic oligonucleotide
  misc_feature 1..33: note = Description of Combined DNA/RNA Molecule: Synthetic oligonucleotide
  modified_base 30..31: mod_base = OTHER; note = 2'-O-methyl modified RNA base
  source 1..33: mol_type = other DNA
  misc_difference 1..33: note = DNA or RNA

SEQ ID NO: 22 - DNA, 33 bp, synthetic construct; identical to SEQ ID NO: 1
  misc_feature 1..33: note = Description of Artificial Sequence: Synthetic oligonucleotide
  misc_feature 1..33: note = Description of Combined DNA/RNA Molecule: Synthetic oligonucleotide
  modified_base 31..32: mod_base = OTHER; note = 2'-O-methyl modified RNA base
  source 1..33: mol_type = other DNA
  misc_difference 1..33: note = DNA or RNA

SEQ ID NO: 23 - DNA, 33 bp, synthetic construct; identical to SEQ ID NO: 1
  misc_feature 1..33: note = Description of Artificial Sequence: Synthetic oligonucleotide
  misc_feature 1..33: note = Description of Combined DNA/RNA Molecule: Synthetic oligonucleotide
  modified_base 32..33: mod_base = OTHER; note = 2'-O-methyl modified RNA base
  source 1..33: mol_type = other DNA
  misc_difference 1..33: note = DNA or RNA

SEQ ID NO: 24 - DNA, 33 bp, synthetic construct; identical to SEQ ID NO: 1
  misc_feature 1..33: note = Description of Artificial Sequence: Synthetic oligonucleotide
  misc_feature 1..33: note = Description of Combined DNA/RNA Molecule: Synthetic oligonucleotide
  modified_base 22..24: mod_base = OTHER; note = 2'-O-methyl modified RNA base
  source 1..33: mol_type = other DNA
  misc_difference 1..33: note = DNA or RNA

SEQ ID NO: 25 - DNA, 33 bp, synthetic construct; identical to SEQ ID NO: 1
  misc_feature 1..33: note = Description of Artificial Sequence: Synthetic oligonucleotide
  misc_feature 1..33: note = Description of Combined DNA/RNA Molecule: Synthetic oligonucleotide
  modified_base 23..25: mod_base = OTHER; note = 2'-O-methyl modified RNA base
  source 1..33: mol_type = other DNA
  misc_difference 1..33: note = DNA or RNA

SEQ ID NO: 26 - DNA, 33 bp, synthetic construct; identical to SEQ ID NO: 1
  misc_feature 1..33: note = Description of Artificial Sequence: Synthetic oligonucleotide
  misc_feature 1..33: note = Description of Combined DNA/RNA Molecule: Synthetic oligonucleotide
  modified_base 24..26: mod_base = OTHER; note = 2'-O-methyl modified RNA base
  source 1..33: mol_type = other DNA
  misc_difference 1..33: note = DNA or RNA

SEQ ID NO: 27 - DNA, 33 bp, synthetic construct; identical to SEQ ID NO: 1
  misc_feature 1..33: note = Description of Artificial Sequence: Synthetic oligonucleotide
  misc_feature 1..33: note = Description of Combined DNA/RNA Molecule: Synthetic oligonucleotide
  modified_base 25..27: mod_base = OTHER; note = 2'-O-methyl modified RNA base
  source 1..33: mol_type = other DNA
  misc_difference 1..33: note = DNA or RNA

SEQ ID NO: 28 - DNA, 33 bp, synthetic construct; identical to SEQ ID NO: 1
  misc_feature 1..33: note = Description of Artificial Sequence: Synthetic oligonucleotide
  misc_feature 1..33: note = Description of Combined DNA/RNA Molecule: Synthetic oligonucleotide
  modified_base 26..28: mod_base = OTHER; note = 2'-O-methyl modified RNA base
  source 1..33: mol_type = other DNA
  misc_difference 1..33: note = DNA or RNA

SEQ ID NO: 29 - DNA, 33 bp, synthetic construct; identical to SEQ ID NO: 1
  misc_feature 1..33: note = Description of Artificial Sequence: Synthetic oligonucleotide
  misc_feature 1..33: note = Description of Combined DNA/RNA Molecule: Synthetic oligonucleotide
  modified_base 27..29: mod_base = OTHER; note = 2'-O-methyl modified RNA base
  source 1..33: mol_type = other DNA
  misc_difference 1..33: note = DNA or RNA

SEQ ID NO: 30 - DNA, 33 bp, synthetic construct; identical to SEQ ID NO: 1
  misc_feature 1..33: note = Description of Artificial Sequence: Synthetic oligonucleotide
  misc_feature 1..33: note = Description of Combined DNA/RNA Molecule: Synthetic oligonucleotide
  modified_base 28..30: mod_base = OTHER; note = 2'-O-methyl modified RNA base
  source 1..33: mol_type = other DNA
  misc_difference 1..33: note = DNA or RNA

SEQ ID NO: 31 - DNA, 33 bp, synthetic construct; identical to SEQ ID NO: 1
  misc_feature 1..33: note = Description of Artificial Sequence: Synthetic oligonucleotide
  misc_feature 1..33: note = Description of Combined DNA/RNA Molecule: Synthetic oligonucleotide
  modified_base 29..31: mod_base = OTHER; note = 2'-O-methyl modified RNA base
  source 1..33: mol_type = other DNA
  misc_difference 1..33: note = DNA or RNA

SEQ ID NO: 32 - DNA, 33 bp, synthetic construct; identical to SEQ ID NO: 1
  misc_feature 1..33: note = Description of Artificial Sequence: Synthetic oligonucleotide
  misc_feature 1..33: note = Description of Combined DNA/RNA Molecule: Synthetic oligonucleotide
  modified_base 30..32: mod_base = OTHER; note = 2'-O-methyl modified RNA base
  source 1..33: mol_type = other DNA
  misc_difference 1..33: note = DNA or RNA

SEQ ID NO: 33 - DNA, 33 bp, synthetic construct; identical to SEQ ID NO: 1
  misc_feature 1..33: note = Description of Artificial Sequence: Synthetic oligonucleotide
  misc_feature 1..33: note = Description of Combined DNA/RNA Molecule: Synthetic oligonucleotide
  modified_base 31..33: mod_base = OTHER; note = 2'-O-methyl modified RNA base
  source 1..33: mol_type = other DNA
  misc_difference 1..33: note = DNA or RNA

SEQ ID NO: 34 - DNA, 33 bp, synthetic construct; identical to SEQ ID NO: 1
  misc_feature 1..33: note = Description of Artificial Sequence: Synthetic oligonucleotide
  misc_feature 1..33: note = Description of Combined DNA/RNA Molecule: Synthetic oligonucleotide
  modified_base 22..25: mod_base = OTHER; note = 2'-O-methyl modified RNA base
  source 1..33: mol_type = other DNA
  misc_difference 1..33: note = DNA or RNA

SEQ ID NO: 35 - DNA, 33 bp, synthetic construct; identical to SEQ ID NO: 1
  misc_feature 1..33: note = Description of Artificial Sequence: Synthetic oligonucleotide
  misc_feature 1..33: note = Description of Combined DNA/RNA Molecule: Synthetic oligonucleotide
  modified_base 23..26: mod_base = OTHER; note = 2'-O-methyl modified RNA base
  source 1..33: mol_type = other DNA
  misc_difference 1..33: note = DNA or RNA

SEQ ID NO: 36 - DNA, 33 bp, synthetic construct; identical to SEQ ID NO: 1
  misc_feature 1..33: note = Description of Artificial Sequence: Synthetic oligonucleotide
  misc_feature 1..33: note = Description of Combined DNA/RNA Molecule: Synthetic oligonucleotide
  modified_base 24..27: mod_base = OTHER; note = 2'-O-methyl modified RNA base
  source 1..33: mol_type = other DNA
  misc_difference 1..33: note = DNA or RNA

SEQ ID NO: 37 - DNA, 33 bp, synthetic construct; identical to SEQ ID NO: 1
  misc_feature 1..33: note = Description of Artificial Sequence: Synthetic oligonucleotide
  misc_feature 1..33: note = Description of Combined DNA/RNA Molecule: Synthetic oligonucleotide
  modified_base 25..28: mod_base = OTHER; note = 2'-O-methyl modified RNA base
  source 1..33: mol_type = other DNA
  misc_difference 1..33: note = DNA or RNA

SEQ ID NO: 38 - DNA, 33 bp, synthetic construct; identical to SEQ ID NO: 1
  misc_feature 1..33: note = Description of Artificial Sequence: Synthetic oligonucleotide
  misc_feature 1..33: note = Description of Combined DNA/RNA Molecule: Synthetic oligonucleotide
  modified_base 26..29: mod_base = OTHER; note = 2'-O-methyl modified RNA base
  source 1..33: mol_type = other DNA
  misc_difference 1..33: note = DNA or RNA

SEQ ID NO: 39 - DNA, 33 bp, synthetic construct; identical to SEQ ID NO: 1
  misc_feature 1..33: note = Description of Artificial Sequence: Synthetic oligonucleotide
  misc_feature 1..33: note = Description of Combined DNA/RNA Molecule: Synthetic oligonucleotide
  modified_base 27..30: mod_base = OTHER; note = 2'-O-methyl modified RNA base
  source 1..33: mol_type = other DNA
  misc_difference 1..33: note = DNA or RNA

SEQ ID NO: 40 - DNA, 33 bp, synthetic construct; identical to SEQ ID NO: 1
  misc_feature 1..33: note = Description of Artificial Sequence: Synthetic oligonucleotide
  misc_feature 1..33: note = Description of Combined DNA/RNA Molecule: Synthetic oligonucleotide
  modified_base 28..31: mod_base = OTHER; note = 2'-O-methyl modified RNA base
  source 1..33: mol_type = other DNA
  misc_difference 1..33: note = DNA or RNA

SEQ ID NO: 41 - DNA, 33 bp, synthetic construct; identical to SEQ ID NO: 1
  misc_feature 1..33: note = Description of Artificial Sequence: Synthetic oligonucleotide
  misc_feature 1..33: note = Description of Combined DNA/RNA Molecule: Synthetic oligonucleotide
  modified_base 29..32: mod_base = OTHER; note = 2'-O-methyl modified RNA base
  source 1..33: mol_type = other DNA
  misc_difference 1..33: note = DNA or RNA

SEQ ID NO: 42 - DNA, 33 bp, synthetic construct; identical to SEQ ID NO: 1
  misc_feature 1..33: note = Description of Artificial Sequence: Synthetic oligonucleotide
  misc_feature 1..33: note = Description of Combined DNA/RNA Molecule: Synthetic oligonucleotide
  modified_base 30..33: mod_base = OTHER; note = 2'-O-methyl modified RNA base
  source 1..33: mol_type = other DNA
  misc_difference 1..33: note = DNA or RNA

SEQ ID NO: 43 - DNA, 33 bp, synthetic construct; identical to SEQ ID NO: 1
  misc_feature 1..33: note = Description of Artificial Sequence: Synthetic oligonucleotide
  misc_feature 1..33: note = Description of Combined DNA/RNA Molecule: Synthetic oligonucleotide
  modified_base 22..26: mod_base = OTHER; note = 2'-O-methyl modified RNA base
  source 1..33: mol_type = other DNA
  misc_difference 1..33: note = DNA or RNA

SEQ ID NO: 44 - DNA, 33 bp, synthetic construct; identical to SEQ ID NO: 1
  misc_feature 1..33: note = Description of Artificial Sequence: Synthetic oligonucleotide
  misc_feature 1..33: note = Description of Combined DNA/RNA Molecule: Synthetic oligonucleotide
  modified_base 23..27: mod_base = OTHER; note = 2'-O-methyl modified RNA base
  source 1..33: mol_type = other DNA
  misc_difference 1..33: note = DNA or RNA

SEQ ID NO: 45 - DNA, 33 bp, synthetic construct; identical to SEQ ID NO: 1
  misc_feature 1..33: note = Description of Artificial Sequence: Synthetic oligonucleotide
  misc_feature 1..33: note = Description of Combined DNA/RNA Molecule: Synthetic oligonucleotide
  modified_base 24..28: mod_base = OTHER; note = 2'-O-methyl modified RNA base
  source 1..33: mol_type = other DNA
  misc_difference 1..33: note = DNA or RNA

SEQ ID NO: 46 - DNA, 33 bp, synthetic construct; identical to SEQ ID NO: 1
  misc_feature 1..33: note = Description of Artificial Sequence: Synthetic oligonucleotide
  misc_feature 1..33: note = Description of Combined DNA/RNA Molecule: Synthetic oligonucleotide
  modified_base 25..29: mod_base = OTHER; note = 2'-O-methyl modified RNA base
  source 1..33: mol_type = other DNA
  misc_difference 1..33: note = DNA or RNA

SEQ ID NO: 47 - DNA, 33 bp, synthetic construct; identical to SEQ ID NO: 1
  misc_feature 1..33: note = Description of Artificial Sequence: Synthetic oligonucleotide
  misc_feature 1..33: note = Description of Combined DNA/RNA Molecule: Synthetic oligonucleotide
  modified_base 26..30: mod_base = OTHER; note = 2'-O-methyl modified RNA base
  source 1..33: mol_type = other DNA
  misc_difference 1..33: note = DNA or RNA

SEQ ID NO: 48 - DNA, 33 bp, synthetic construct; identical to SEQ ID NO: 1
  misc_feature 1..33: note = Description of Artificial Sequence: Synthetic oligonucleotide
  misc_feature 1..33: note = Description of Combined DNA/RNA Molecule: Synthetic oligonucleotide
  modified_base 27..31: mod_base = OTHER; note = 2'-O-methyl modified RNA base
  source 1..33: mol_type = other DNA
  misc_difference 1..33: note = DNA or RNA

SEQ ID NO: 49 - DNA, 33 bp, synthetic construct; identical to SEQ ID NO: 1
  misc_feature 1..33: note = Description of Artificial Sequence: Synthetic oligonucleotide
  misc_feature 1..33: note = Description of Combined DNA/RNA Molecule: Synthetic oligonucleotide
  modified_base 28..32: mod_base = OTHER; note = 2'-O-methyl modified RNA base
  source 1..33: mol_type = other DNA
  misc_difference 1..33: note = DNA or RNA

SEQ ID NO: 50 - DNA, 33 bp, synthetic construct; identical to SEQ ID NO: 1
  misc_feature 1..33: note = Description of Artificial Sequence: Synthetic oligonucleotide
  misc_feature 1..33: note = Description of Combined DNA/RNA Molecule: Synthetic oligonucleotide
  modified_base 29..33: mod_base = OTHER; note = 2'-O-methyl modified RNA base
  source 1..33: mol_type = other DNA
  misc_difference 1..33: note = DNA or RNA

SEQ ID NO: 51 - DNA, 33 bp, synthetic construct; identical to SEQ ID NO: 1
  misc_feature 1..33: note = Description of Artificial Sequence: Synthetic oligonucleotide
  misc_feature 1..33: note = Description of Combined DNA/RNA Molecule: Synthetic oligonucleotide
  modified_base 22..33: mod_base = OTHER; note = 2'-O-methyl modified RNA base
  source 1..33: mol_type = other DNA
  misc_difference 1..33: note = DNA or RNA

SEQ ID NO: 52 - DNA, 33 bp, synthetic construct; identical to SEQ ID NO: 1
  misc_feature 1..33: note = Description of Artificial Sequence: Synthetic oligonucleotide
  misc_feature 1..33: note = Description of Combined DNA/RNA Molecule: Synthetic oligonucleotide
  modified_base 23..33: mod_base = OTHER; note = 2'-O-methyl modified RNA base
  source 1..33: mol_type = other DNA
  misc_difference 1..33: note = DNA or RNA

SEQ ID NO: 53 - DNA, 33 bp, synthetic construct; identical to SEQ ID NO: 1
  misc_feature 1..33: note = Description of Artificial Sequence: Synthetic oligonucleotide
  misc_feature 1..33: note = Description of Combined DNA/RNA Molecule: Synthetic oligonucleotide
  modified_base 24..33: mod_base = OTHER; note = 2'-O-methyl modified RNA base
  source 1..33: mol_type = other DNA
  misc_difference 1..33: note = DNA or RNA

SEQ ID NO: 54 - DNA, 33 bp, synthetic construct; identical to SEQ ID NO: 1
  misc_feature 1..33: note = Description of Artificial Sequence: Synthetic oligonucleotide
  misc_feature 1..33: note = Description of Combined DNA/RNA Molecule: Synthetic oligonucleotide
  modified_base 25..33: mod_base = OTHER; note = 2'-O-methyl modified RNA base
  source 1..33: mol_type = other DNA
  misc_difference 1..33: note = DNA or RNA

SEQ ID NO: 55 - DNA, 33 bp, synthetic construct; identical to SEQ ID NO: 1
  misc_feature 1..33: note = Description of Artificial Sequence: Synthetic oligonucleotide
  misc_feature 1..33: note = Description of Combined DNA/RNA Molecule: Synthetic oligonucleotide
  modified_base 26..33: mod_base = OTHER; note = 2'-O-methyl modified RNA base
  source 1..33: mol_type = other DNA
  misc_difference 1..33: note = DNA or RNA

SEQ ID NO: 56 - DNA, 33 bp, synthetic construct; identical to SEQ ID NO: 1
  misc_feature 1..33: note = Description of Artificial Sequence: Synthetic oligonucleotide
  misc_feature 1..33: note = Description of Combined DNA/RNA Molecule: Synthetic oligonucleotide
  modified_base 27..33: mod_base = OTHER; note = 2'-O-methyl modified RNA base
  source 1..33: mol_type = other DNA
  misc_difference 1..33: note = DNA or RNA

SEQ ID NO: 57 - DNA, 33 bp, synthetic construct; identical to SEQ ID NO: 1
  misc_feature 1..33: note = Description of Artificial Sequence: Synthetic oligonucleotide
  misc_feature 1..33: note = Description of Combined DNA/RNA Molecule: Synthetic oligonucleotide
  modified_base 28..33: mod_base = OTHER; note = 2'-O-methyl modified RNA base
  source 1..33: mol_type = other DNA
  misc_difference 1..33: note = DNA or RNA

SEQ ID NO: 58 - DNA, 29 bp, synthetic construct
  misc_feature 1..29: note = Description of Artificial Sequence: Synthetic primer
  misc_feature 1..29: note = Description of Combined DNA/RNA Molecule: Synthetic primer
  modified_base 18: mod_base = OTHER; note = 2'-O-methyl modified RNA base
  modified_base 20: mod_base = OTHER; note = 2'-O-methyl modified RNA base
  modified_base 22: mod_base = OTHER; note = 2'-O-methyl modified RNA base
  modified_base 24..28: mod_base = OTHER; note = 2'-O-methyl modified RNA base
  source 1..29: mol_type = other DNA
  misc_difference 1..29: note = DNA or RNA
cgcggagtcctcgaactataagccacgca

SEQ ID NO: 59 - DNA, 32 bp, synthetic construct
  misc_feature 1..32: note = Description of Artificial Sequence: Synthetic primer
  misc_feature 1..32: note = Description of Combined DNA/RNA Molecule: Synthetic primer
  modified_base 19: mod_base = OTHER; note = 2'-O-methyl modified RNA base
  modified_base 21: mod_base = OTHER; note = 2'-O-methyl modified RNA base
  modified_base 23: mod_base = OTHER; note = 2'-O-methyl modified RNA base
  modified_base 25: mod_base = OTHER; note = 2'-O-methyl modified RNA base
  modified_base 27..31: mod_base = OTHER; note = 2'-O-methyl modified RNA base
  source 1..32: mol_type = other DNA
  misc_difference 1..32: note = DNA or RNA
cgcggagtccgcgtgtacagctccaccacatt

SEQ ID NO: 60 - DNA, 29 bp, synthetic construct
  misc_feature 1..29: note = Description of Artificial Sequence: Synthetic primer
  misc_feature 1..29: note = Description of Combined DNA/RNA Molecule: Synthetic primer
  modified_base 24..29: mod_base = OTHER; note = 2'-O-methyl modified RNA base
  source 1..29: mol_type = other DNA
  misc_difference 1..29: note = DNA or RNA
cgcggagtcctcgaactataagccacgca

SEQ ID NO: 61 - DNA, 32 bp, synthetic construct; identical to SEQ ID NO: 59
  misc_feature 1..32: note = Description of Artificial Sequence: Synthetic primer
  misc_feature 1..32: note = Description of Combined DNA/RNA Molecule: Synthetic primer
  modified_base 27..32: mod_base = OTHER; note = 2'-O-methyl modified RNA base
  source 1..32: mol_type = other DNA
  misc_difference 1..32: note = DNA or RNA